European Patent Application EP 4 592 318 A1, published July 30, 2025. Title: 人源化的L1CAM抗体药物偶联物. Applicant: 同润生物医药(上海)有限公司. The sequence listing filed with the application follows.

SEQUENCE LISTING (56 sequences)

SEQ ID NO: 1 - protein, 8 aa, synthetic construct
GYTFTNYW

SEQ ID NO: 2 - protein, 8 aa, synthetic construct
INPSTYYS

SEQ ID NO: 3 - protein, 12 aa, synthetic construct
ARRQFGLPLFDY

SEQ ID NO: 4 - protein, 6 aa, synthetic construct
QDVGTA

SEQ ID NO: 5 - skipped

SEQ ID NO: 6 - protein, 9 aa, synthetic construct
QQYSNYPLT

SEQ ID NO: 7 - protein, 8 aa, synthetic construct
GYTFTRYW

SEQ ID NO: 8 - protein, 8 aa, synthetic construct
INPSTGYT

SEQ ID NO: 9 - protein, 12 aa, synthetic construct
ARRHLGLPLFDY

SEQ ID NO: 10 - protein, 9 aa, synthetic construct
GGSISSDYA

SEQ ID NO: 11 - protein, 7 aa, synthetic construct
ITYSGTT

SEQ ID NO: 12 - protein, 13 aa, synthetic construct
ARDHYGNYAYFDY

SEQ ID NO: 13 - protein, 5 aa, synthetic construct
SSVSF

SEQ ID NO: 14 - skipped

SEQ ID NO: 15 - protein, 9 aa, synthetic construct
QQWSSNPST

SEQ ID NO: 16 - protein, 8 aa, synthetic construct
GYTFTSYT

SEQ ID NO: 17 - protein, 7 aa, synthetic construct
INPNYGG

SEQ ID NO: 18 - protein, 13 aa, synthetic construct
AREGATGTWYFDV

SEQ ID NO: 19 - skipped

SEQ ID NO: 20 - protein, 9 aa, synthetic construct
QQWRSNPPT

SEQ ID NO: 21 - protein, 119 aa, synthetic construct
QVQLVQSGAEVKKPGSSVKVSCKASGYTFTNYWIQWVRQAPGQGLEWIGYINPSTYYSDYNQKFQGRVTLTADKSTSTAYMELSSLRSEDTAVYYCARRQFGLPLFDYWGQGTTVTVSS

SEQ ID NO: 22 - protein, 107 aa, synthetic construct
DIQMTQSPSSLSASVGDRVTITCRASQDVGTAVAWYQQKPGKVPKLLIYWASTLHSGVPSRFSGSGSGTDFTLTISSLQPEDVATYFCQQYSNYPLTFGGGTKVEIK

SEQ ID NO: 23 - protein, 119 aa, synthetic construct
QVQLVQSGAEVKKPGSSVKVSCKASGYTFTRYWIQWVRQAPGQGLEWMGYINPSTGYTDYNQKFQGRVTITADKSTSTAYMELSSLRSEDTAVYYCARRHLGLPLFDYWGQGTTVTVSS

SEQ ID NO: 24 - protein, 107 aa, synthetic construct
DIQMTQSPSSVSASVGDRVTITCRASQDVGTAVAWYQQKPGKAPKLLIYWASSLHSGVPSRFSGSGSGTDFTLTISSLQPEDFATYFCQQYSNYPLTFGGGTKVEIK

SEQ ID NO: 25 - protein, 120 aa, synthetic construct
DVQLQESGPGLVKPSQTLSLTCTVSGGSISSDYAWNWIRQPPGKGLEWMGYITYSGTTTYNPSLKSRITISRDTSKNQFSLKLSSVTAADTAVYYCARDHYGNYAYFDYWGQGTTVTVSS

SEQ ID NO: 26 - protein, 106 aa, synthetic construct
DIQMTQSPSSLSASVGDRVTITCRASSSVSFMHWYQQKPGKAPKPWIYASSNLVSGVPSRFSGSGSGTDFTLTISSLQPEDFATYYCQQWSSNPSTFGGGTKVEIK

SEQ ID NO: 27 - protein, 120 aa, synthetic construct; identical to SEQ ID NO: 25

SEQ ID NO: 28 - protein, 106 aa, synthetic construct
QIQMTQSPSSLSASVGDRVTITCRASSSVSFMHWYQQKPGKAPKPWIYASSNLVSGVPSRFSGSGSGTDYTLTISSLQPEDFATYYCQQWSSNPSTFGGGTKVEIK

SEQ ID NO: 29 - protein, 120 aa, synthetic construct
EVQLVQSGAEVKKPGASVKVSCKASGYTFTSYTMHWVRQAPGQGLEWMGDINPNYGGTSYNEKFKDRVTMTTDTSTSTAYMELRSLRSDDTAVYYCAREGATGTWYFDVWGQGTTVTVSS

SEQ ID NO: 30 - protein, 106 aa, synthetic construct
DIQMTQSPSSLSASVGDRVTITCSASSSVSFMFWYQQKPGKAPKPLIYLTSNLASGVPSRFSGSGSGTDFTLTISSLQPEDFATYYCQQWRSNPPTFGGGTKVEIK

SEQ ID NO: 31 - protein, 120 aa, synthetic construct
EVQLVQSGAEVKKPGASVKVSCKASGYTFTSYTMHWVRQAPGQGLEWMGDINPNYGGTSYNEKFKDRATMTTDTSTSTAYMELRSLRSDDTAVYYCAREGATGTWYFDVWGQGTTVTVSS

SEQ ID NO: 32 - protein, 106 aa, synthetic construct; identical to SEQ ID NO: 30

SEQ ID NO: 33 - protein, 449 aa, synthetic construct
QVQLVQSGAEVKKPGSSVKVSCKASGYTFTNYWIQWVRQAPGQGLEWIGYINPSTYYSDYNQKFQGRVTLTADKSTSTAYMELSSLRSEDTAVYYCARRQFGLPLFDYWGQGTTVTVSSASTKGPSVFPLAPSSKSTSGGTAALGCLVKDYFPEPVTVSWNSGALTSGVHTFPAVLQSSGLYSLSSVVTVPSSSLGTQTYICNVNHKPSNTKVDKKVEPKSCDKTHTCPPCPAPELLGGPSVFLFPPKPKDTLMISRTPEVTCVVVDVSHEDPEVKFNWYVDGVEVHNAKTKPREEQYNSTYRVVSVLTVLHQDWLNGKEYKCKVSNKALPAPIEKTISKAKGQPREPQVYTLPPSREEMTKNQVSLTCLVKGFYPSDIAVEWESNGQPENNYKTTPPVLDSDGSFFLYSKLTVDKSRWQQGNVFSCSVMHEALHNHYTQKSLSLSPGK

SEQ ID NO: 34 - protein, 214 aa, synthetic construct
DIQMTQSPSSLSASVGDRVTITCRASQDVGTAVAWYQQKPGKVPKLLIYWASTLHSGVPSRFSGSGSGTDFTLTISSLQPEDVATYFCQQYSNYPLTFGGGTKVEIKRTVAAPSVFIFPPSDEQLKSGTASVVCLLNNFYPREAKVQWKVDNALQSGNSQESVTEQDSKDSTYSLSSTLTLSKADYEKHKVYACEVTHQGLSSPVTKSFNRGEC

SEQ ID NO: 35 - protein, 449 aa, synthetic construct
QVQLVQSGAEVKKPGSSVKVSCKASGYTFTRYWIQWVRQAPGQGLEWMGYINPSTGYTDYNQKFQGRVTITADKSTSTAYMELSSLRSEDTAVYYCARRHLGLPLFDYWGQGTTVTVSSASTKGPSVFPLAPSSKSTSGGTAALGCLVKDYFPEPVTVSWNSGALTSGVHTFPAVLQSSGLYSLSSVVTVPSSSLGTQTYICNVNHKPSNTKVDKKVEPKSCDKTHTCPPCPAPELLGGPSVFLFPPKPKDTLMISRTPEVTCVVVDVSHEDPEVKFNWYVDGVEVHNAKTKPREEQYNSTYRVVSVLTVLHQDWLNGKEYKCKVSNKALPAPIEKTISKAKGQPREPQVYTLPPSREEMTKNQVSLTCLVKGFYPSDIAVEWESNGQPENNYKTTPPVLDSDGSFFLYSKLTVDKSRWQQGNVFSCSVMHEALHNHYTQKSLSLSPGK

SEQ ID NO: 36 - protein, 214 aa, synthetic construct
DIQMTQSPSSVSASVGDRVTITCRASQDVGTAVAWYQQKPGKAPKLLIYWASSLHSGVPSRFSGSGSGTDFTLTISSLQPEDFATYFCQQYSNYPLTFGGGTKVEIKRTVAAPSVFIFPPSDEQLKSGTASVVCLLNNFYPREAKVQWKVDNALQSGNSQESVTEQDSKDSTYSLSSTLTLSKADYEKHKVYACEVTHQGLSSPVTKSFNRGEC

SEQ ID NO: 37 - protein, 450 aa, synthetic construct
DVQLQESGPGLVKPSQTLSLTCTVSGGSISSDYAWNWIRQPPGKGLEWMGYITYSGTTTYNPSLKSRITISRDTSKNQFSLKLSSVTAADTAVYYCARDHYGNYAYFDYWGQGTTVTVSSASTKGPSVFPLAPSSKSTSGGTAALGCLVKDYFPEPVTVSWNSGALTSGVHTFPAVLQSSGLYSLSSVVTVPSSSLGTQTYICNVNHKPSNTKVDKKVEPKSCDKTHTCPPCPAPELLGGPSVFLFPPKPKDTLMISRTPEVTCVVVDVSHEDPEVKFNWYVDGVEVHNAKTKPREEQYNSTYRVVSVLTVLHQDWLNGKEYKCKVSNKALPAPIEKTISKAKGQPREPQVYTLPPSREEMTKNQVSLTCLVKGFYPSDIAVEWESNGQPENNYKTTPPVLDSDGSFFLYSKLTVDKSRWQQGNVFSCSVMHEALHNHYTQKSLSLSPGK

SEQ ID NO: 38 - protein, 213 aa, synthetic construct
DIQMTQSPSSLSASVGDRVTITCRASSSVSFMHWYQQKPGKAPKPWIYASSNLVSGVPSRFSGSGSGTDFTLTISSLQPEDFATYYCQQWSSNPSTFGGGTKVEIKRTVAAPSVFIFPPSDEQLKSGTASVVCLLNNFYPREAKVQWKVDNALQSGNSQESVTEQDSKDSTYSLSSTLTLSKADYEKHKVYACEVTHQGLSSPVTKSFNRGEC

SEQ ID NO: 39 - protein, 450 aa, synthetic construct; identical to SEQ ID NO: 37

SEQ ID NO: 40 - protein, 213 aa, synthetic construct
QIQMTQSPSSLSASVGDRVTITCRASSSVSFMHWYQQKPGKAPKPWIYASSNLVSGVPSRFSGSGSGTDYTLTISSLQPEDFATYYCQQWSSNPSTFGGGTKVEIKRTVAAPSVFIFPPSDEQLKSGTASVVCLLNNFYPREAKVQWKVDNALQSGNSQESVTEQDSKDSTYSLSSTLTLSKADYEKHKVYACEVTHQGLSSPVTKSFNRGEC

SEQ ID NO: 41 - protein, 450 aa, synthetic construct
EVQLVQSGAEVKKPGASVKVSCKASGYTFTSYTMHWVRQAPGQGLEWMGDINPNYGGTSYNEKFKDRVTMTTDTSTSTAYMELRSLRSDDTAVYYCAREGATGTWYFDVWGQGTTVTVSSASTKGPSVFPLAPSSKSTSGGTAALGCLVKDYFPEPVTVSWNSGALTSGVHTFPAVLQSSGLYSLSSVVTVPSSSLGTQTYICNVNHKPSNTKVDKKVEPKSCDKTHTCPPCPAPELLGGPSVFLFPPKPKDTLMISRTPEVTCVVVDVSHEDPEVKFNWYVDGVEVHNAKTKPREEQYNSTYRVVSVLTVLHQDWLNGKEYKCKVSNKALPAPIEKTISKAKGQPREPQVYTLPPSREEMTKNQVSLTCLVKGFYPSDIAVEWESNGQPENNYKTTPPVLDSDGSFFLYSKLTVDKSRWQQGNVFSCSVMHEALHNHYTQKSLSLSPGK

SEQ ID NO: 42 - protein, 213 aa, synthetic construct
DIQMTQSPSSLSASVGDRVTITCSASSSVSFMFWYQQKPGKAPKPLIYLTSNLASGVPSRFSGSGSGTDFTLTISSLQPEDFATYYCQQWRSNPPTFGGGTKVEIKRTVAAPSVFIFPPSDEQLKSGTASVVCLLNNFYPREAKVQWKVDNALQSGNSQESVTEQDSKDSTYSLSSTLTLSKADYEKHKVYACEVTHQGLSSPVTKSFNRGEC

SEQ ID NO: 43 - protein, 450 aa, synthetic construct
EVQLVQSGAEVKKPGASVKVSCKASGYTFTSYTMHWVRQAPGQGLEWMGDINPNYGGTSYNEKFKDRATMTTDTSTSTAYMELRSLRSDDTAVYYCAREGATGTWYFDVWGQGTTVTVSSASTKGPSVFPLAPSSKSTSGGTAALGCLVKDYFPEPVTVSWNSGALTSGVHTFPAVLQSSGLYSLSSVVTVPSSSLGTQTYICNVNHKPSNTKVDKKVEPKSCDKTHTCPPCPAPELLGGPSVFLFPPKPKDTLMISRTPEVTCVVVDVSHEDPEVKFNWYVDGVEVHNAKTKPREEQYNSTYRVVSVLTVLHQDWLNGKEYKCKVSNKALPAPIEKTISKAKGQPREPQVYTLPPSREEMTKNQVSLTCLVKGFYPSDIAVEWESNGQPENNYKTTPPVLDSDGSFFLYSKLTVDKSRWQQGNVFSCSVMHEALHNHYTQKSLSLSPGK

SEQ ID NO: 44 - protein, 213 aa, synthetic construct; identical to SEQ ID NO: 42

SEQ ID NO: 45 - DNA, 1347 bp, synthetic construct
  source 1..1347: mol_type = other DNA
caggtccaactcgtccaaagcggcgcagaagtcaaaaaacccggcagctcagtcaaagttagctgcaaggccagcggctacaccttcacaaactactggattcaatgggtgagacaagccccaggccaagggctcgaatggataggctacatcaaccccagcacctactatagcgactacaaccagaaattccagggcagagtcaccctgaccgccgacaaaagcaccagcaccgcttacatggaactgtccagcctgagaagcgaggacaccgccgtgtactactgcgccagaagacaattcggactgcccctgttcgattactggggccagggaaccaccgtgaccgtgagcagcgctagcaccaagggcccatcggtcttccccctggcaccctcctccaagagcacctctgggggcacagcggccctgggctgcctggtcaaggactacttccccgaaccggtgacggtgtcgtggaactcaggcgccctgaccagcggcgtgcacaccttcccggctgtcctacagtcctcaggactctactccctcagcagcgtggtgaccgtgccctccagcagcttgggcacccagacctacatctgcaacgtgaatcacaagcccagcaacaccaaggtggacaagaaagttgagcccaaatcttgtgacaaaactcacacatgcccaccgtgcccagcacctgaactcctggggggaccgtcagtcttcctcttccccccaaaacccaaggacaccctcatgatctcccggacccccgaggtcacatgcgtggtggtggacgtgagccacgaagaccctgaggtcaagttcaactggtacgtggacggcgtggaggtgcataatgccaagacaaagccgcgggaggagcagtacaacagcacgtaccgtgtggtcagcgtcctcaccgtcctgcaccaggactggctgaatggcaaggagtacaagtgcaaggtctccaacaaagccctcccagcccccatcgagaaaaccatctccaaagccaaagggcagccccgagaaccacaggtgtacaccctgcccccatcccgggaggagatgaccaagaaccaggtcagcctgacctgcctggtcaaaggcttctatcccagcgacatcgccgtggagtgggagagcaatgggcagccggagaacaactacaagaccacgcctcccgtgctggactccgacggctccttcttcctctacagcaagctcaccgtggacaagagcaggtggcagcaggggaacgtcttctcatgctccgtgatgcatgaggctctgcacaaccactacacgcagaagagcctctccctgtctccgggtaaa

SEQ ID NO: 46 - DNA, 642 bp, synthetic construct
  source 1..642: mol_type = other DNA
gacattcagatgacccagagccccagcagcctgagcgccagcgtgggagacagagtgaccataacctgcagagccagccaagacgttggaaccgccgtggcctggtatcagcagaaacccggaaaggtgcccaaactgctgatctactgggccagcaccctgcattccggagtgcccagcagattcagcggaagcggaagcgggacagacttcaccctgaccatcagcagcctgcaaccagaggacgtcgccacctacttctgccagcagtacagcaactaccccctgaccttcggaggcggcacaaaagtcgaaatcaagcgtacggtggctgcaccatctgtcttcatcttcccgccatctgatgagcagttgaaatctggaactgcctctgttgtgtgcctgctgaataacttctatcccagagaggccaaagtacagtggaaggtggataacgccctccaatcgggtaactcccaggagagtgtcacagagcaggacagcaaggacagcacctacagcctcagcagcaccctgacgctgagcaaagcagactacgagaaacacaaagtctacgcctgcgaagtcacccatcagggcctgagttcgcccgtcacaaagagcttcaacaggggagagtgt

SEQ ID NO: 47 - DNA, 1347 bp, synthetic construct
  source 1..1347: mol_type = other DNA
caggtccaactcgtccaaagcggcgcagaagtcaaaaaacccggcagctcagtcaaagttagctgcaaggccagcggctacaccttcacaagatactggattcaatgggtgagacaagccccaggccaagggctcgaatggatgggatacatcaacccctcaaccggctacaccgactacaaccagaagttccagggcagagtgaccatcaccgccgacaaaagcacaagcaccgcctacatggagctgtccagcctgcgcagcgaggacaccgccgtctactattgcgccagaagacacctcggcctgcccctgttcgattactggggccaaggaaccacagtgaccgtgagtagcgctagcaccaagggcccatcggtcttccccctggcaccctcctccaagagcacctctgggggcacagcggccctgggctgcctggtcaaggactacttccccgaaccggtgacggtgtcgtggaactcaggcgccctgaccagcggcgtgcacaccttcccggctgtcctacagtcctcaggactctactccctcagcagcgtggtgaccgtgccctccagcagcttgggcacccagacctacatctgcaacgtgaatcacaagcccagcaacaccaaggtggacaagaaagttgagcccaaatcttgtgacaaaactcacacatgcccaccgtgcccagcacctgaactcctggggggaccgtcagtcttcctcttccccccaaaacccaaggacaccctcatgatctcccggacccccgaggtcacatgcgtggtggtggacgtgagccacgaagaccctgaggtcaagttcaactggtacgtggacggcgtggaggtgcataatgccaagacaaagccgcgggaggagcagtacaacagcacgtaccgtgtggtcagcgtcctcaccgtcctgcaccaggactggctgaatggcaaggagtacaagtgcaaggtctccaacaaagccctcccagcccccatcgagaaaaccatctccaaagccaaagggcagccccgagaaccacaggtgtacaccctgcccccatcccgggaggagatgaccaagaaccaggtcagcctgacctgcctggtcaaaggcttctatcccagcgacatcgccgtggagtgggagagcaatgggcagccggagaacaactacaagaccacgcctcccgtgctggactccgacggctccttcttcctctacagcaagctcaccgtggacaagagcaggtggcagcaggggaacgtcttctcatgctccgtgatgcatgaggctctgcacaaccactacacgcagaagagcctctccctgtctccgggtaaa

SEQ ID NO: 48 - DNA, 642 bp, synthetic construct
  source 1..642: mol_type = other DNA
gacattcagatgacccagagccccagcagcgtgagcgccagcgtgggagacagagtgaccataacctgcagagccagccaagacgttggaaccgccgtggcctggtatcagcagaaacccggaaaggcccccaaactgctcatctactgggcaagcagcctgcacagcggagtgcccagcagatttagcggaagcggaagcgggacagactttaccctgaccatcagcagcctccaacctgaggatttcgccacctacttctgccagcaatacagcaactacccactgaccttcggaggcggcacaaaagtcgagatcaagcgtacggtggctgcaccatctgtcttcatcttcccgccatctgatgagcagttgaaatctggaactgcctctgttgtgtgcctgctgaataacttctatcccagagaggccaaagtacagtggaaggtggataacgccctccaatcgggtaactcccaggagagtgtcacagagcaggacagcaaggacagcacctacagcctcagcagcaccctgacgctgagcaaagcagactacgagaaacacaaagtctacgcctgcgaagtcacccatcagggcctgagttcgcccgtcacaaagagcttcaacaggggagagtgt

SEQ ID NO: 49 - DNA, 1350 bp, synthetic construct
  source 1..1350: mol_type = other DNA
gacgtgcagctgcaagagagcggacccggactggtgaagcccagccaaacactgagcctgacatgcacagtgagcggaggaagcataagcagcgactacgcctggaactggattagacagccccccggcaagggcctggagtggatgggatatatcacctacagcggcaccaccacctacaatcccagcctgaaaagcagaatcaccatctccagggacaccagcaagaaccagttcagcctcaagctgagcagcgtgaccgccgccgacaccgcagtctactactgcgcccgagaccactacggaaactacgcctacttcgactactggggccagggcaccaccgtgaccgtgtccagcgctagcaccaagggcccatcggtcttccccctggcaccctcctccaagagcacctctgggggcacagcggccctgggctgcctggtcaaggactacttccccgaaccggtgacggtgtcgtggaactcaggcgccctgaccagcggcgtgcacaccttcccggctgtcctacagtcctcaggactctactccctcagcagcgtggtgaccgtgccctccagcagcttgggcacccagacctacatctgcaacgtgaatcacaagcccagcaacaccaaggtggacaagaaagttgagcccaaatcttgtgacaaaactcacacatgcccaccgtgcccagcacctgaactcctggggggaccgtcagtcttcctcttccccccaaaacccaaggacaccctcatgatctcccggacccccgaggtcacatgcgtggtggtggacgtgagccacgaagaccctgaggtcaagttcaactggtacgtggacggcgtggaggtgcataatgccaagacaaagccgcgggaggagcagtacaacagcacgtaccgtgtggtcagcgtcctcaccgtcctgcaccaggactggctgaatggcaaggagtacaagtgcaaggtctccaacaaagccctcccagcccccatcgagaaaaccatctccaaagccaaagggcagccccgagaaccacaggtgtacaccctgcccccatcccgggaggagatgaccaagaaccaggtcagcctgacctgcctggtcaaaggcttctatcccagcgacatcgccgtggagtgggagagcaatgggcagccggagaacaactacaagaccacgcctcccgtgctggactccgacggctccttcttcctctacagcaagctcaccgtggacaagagcaggtggcagcaggggaacgtcttctcatgctccgtgatgcatgaggctctgcacaaccactacacgcagaagagcctctccctgtctccgggtaaa

SEQ ID NO: 50 - DNA, 639 bp, synthetic construct
  source 1..639: mol_type = other DNA
gacattcagatgacccagagccccagcagcctgagcgccagcgtgggagacagagtgaccataacctgcagagccagcagcagcgttagcttcatgcactggtaccagcagaaacccggcaaggcccccaaaccctggatctacgcctccagcaacctggtgagcggagtgccaagcagattcagcggcagcggcagcggaaccgacttcaccctcactatcagcagcctccaacccgaagacttcgccacctactactgccagcagtggagctccaatcccagcaccttcggcggcggcacaaaggtggagatcaaacgtacggtggctgcaccatctgtcttcatcttcccgccatctgatgagcagttgaaatctggaactgcctctgttgtgtgcctgctgaataacttctatcccagagaggccaaagtacagtggaaggtggataacgccctccaatcgggtaactcccaggagagtgtcacagagcaggacagcaaggacagcacctacagcctcagcagcaccctgacgctgagcaaagcagactacgagaaacacaaagtctacgcctgcgaagtcacccatcagggcctgagttcgcccgtcacaaagagcttcaacaggggagagtgt

SEQ ID NO: 51 - DNA, 1350 bp, synthetic construct; identical to SEQ ID NO: 49
  source 1..1350: mol_type = other DNA

SEQ ID NO: 52 - DNA, 639 bp, synthetic construct
  source 1..639: mol_type = other DNA
cagatccaaatgacccaaagccccagcagcctctccgccagcgtcggagacagagtcaccatcacctgcagagccagcagcagcgtctccttcatgcactggtaccaacagaaacccggcaaggcccccaagccctggatctacgcctcctccaatctggtgtcaggagtgcccagcagattcagcggcagcggcagcggaaccgactacaccctcactatcagcagcctccaacctgaagatttcgccacctattactgccaacagtggagcagcaaccccagcaccttcggaggcggtaccaaggtcgaaatcaaacgtacggtggctgcaccatctgtcttcatcttcccgccatctgatgagcagttgaaatctggaactgcctctgttgtgtgcctgctgaataacttctatcccagagaggccaaagtacagtggaaggtggataacgccctccaatcgggtaactcccaggagagtgtcacagagcaggacagcaaggacagcacctacagcctcagcagcaccctgacgctgagcaaagcagactacgagaaacacaaagtctacgcctgcgaagtcacccatcagggcctgagttcgcccgtcacaaagagcttcaacaggggagagtgt

SEQ ID NO: 53 - DNA, 1350 bp, synthetic construct
  source 1..1350: mol_type = other DNA
gaggtgcagctggtgcagagcggagcagaggtgaagaagccaggggccagcgtgaaggtgagctgtaaggctagtgggtacacatttacaagctacacaatgcactgggtgagacaggccccaggccaaggactggagtggatgggagacataaaccccaattacggaggaacaagctacaacgaaaaattcaaagacagagtgaccatgaccaccgacacaagcacaagcaccgcctacatggagctgagaagtctgagatcagacgacaccgccgtctactactgcgccagagagggagccaccgggacctggtacttcgacgtgtggggccagggaacaacagtgaccgtgagcagcgctagcaccaagggcccatcggtcttccccctggcaccctcctccaagagcacctctgggggcacagcggccctgggctgcctggtcaaggactacttccccgaaccggtgacggtgtcgtggaactcaggcgccctgaccagcggcgtgcacaccttcccggctgtcctacagtcctcaggactctactccctcagcagcgtggtgaccgtgccctccagcagcttgggcacccagacctacatctgcaacgtgaatcacaagcccagcaacaccaaggtggacaagaaagttgagcccaaatcttgtgacaaaactcacacatgcccaccgtgcccagcacctgaactcctggggggaccgtcagtcttcctcttccccccaaaacccaaggacaccctcatgatctcccggacccccgaggtcacatgcgtggtggtggacgtgagccacgaagaccctgaggtcaagttcaactggtacgtggacggcgtggaggtgcataatgccaagacaaagccgcgggaggagcagtacaacagcacgtaccgtgtggtcagcgtcctcaccgtcctgcaccaggactggctgaatggcaaggagtacaagtgcaaggtctccaacaaagccctcccagcccccatcgagaaaaccatctccaaagccaaagggcagccccgagaaccacaggtgtacaccctgcccccatcccgggaggagatgaccaagaaccaggtcagcctgacctgcctggtcaaaggcttctatcccagcgacatcgccgtggagtgggagagcaatgggcagccggagaacaactacaagaccacgcctcccgtgctggactccgacggctccttcttcctctacagcaagctcaccgtggacaagagcaggtggcagcaggggaacgtcttctcatgctccgtgatgcatgaggctctgcacaaccactacacgcagaagagcctctccctgtctccgggtaaa

SEQ ID NO: 54 - DNA, 639 bp, synthetic construct
  source 1..639: mol_type = other DNA
gacattcagatgacccagagccccagcagcctgagcgccagcgtgggagacagagtgaccataacctgcagcgccagctccagcgtgagcttcatgttttggtaccagcagaaacccggcaaggcccccaagcccctgatatacctgaccagcaacctggcctctggagtgcccagccggttctccggaagcggctctggaactgacttcaccctcaccatctccagcctgcaacccgaagacttcgccacctactactgccagcaatggagatccaatccccccaccttcggcggcggcaccaaggttgagatcaaacgtacggtggctgcaccatctgtcttcatcttcccgccatctgatgagcagttgaaatctggaactgcctctgttgtgtgcctgctgaataacttctatcccagagaggccaaagtacagtggaaggtggataacgccctccaatcgggtaactcccaggagagtgtcacagagcaggacagcaaggacagcacctacagcctcagcagcaccctgacgctgagcaaagcagactacgagaaacacaaagtctacgcctgcgaagtcacccatcagggcctgagttcgcccgtcacaaagagcttcaacaggggagagtgt

SEQ ID NO: 55 - DNA, 1350 bp, synthetic construct
  source 1..1350: mol_type = other DNA
gaggtgcagctggtgcagagcggagcagaggtgaagaagccaggggccagcgtgaaggtgagctgtaaggctagtgggtacacatttacaagctacacaatgcactgggtgagacaggccccaggccaaggactggagtggatgggagacataaaccccaattacggaggaacaagctacaacgaaaaattcaaagacagagccacaatgaccacagacaccagcaccagcaccgcatacatggaactgagaagcctcaggagcgacgacaccgcagtgtactactgcgccagagagggagccaccgggacctggtacttcgacgtgtggggccagggcaccaccgtgaccgtgagcagcgctagcaccaagggcccatcggtcttccccctggcaccctcctccaagagcacctctgggggcacagcggccctgggctgcctggtcaaggactacttccccgaaccggtgacggtgtcgtggaactcaggcgccctgaccagcggcgtgcacaccttcccggctgtcctacagtcctcaggactctactccctcagcagcgtggtgaccgtgccctccagcagcttgggcacccagacctacatctgcaacgtgaatcacaagcccagcaacaccaaggtggacaagaaagttgagcccaaatcttgtgacaaaactcacacatgcccaccgtgcccagcacctgaactcctggggggaccgtcagtcttcctcttccccccaaaacccaaggacaccctcatgatctcccggacccccgaggtcacatgcgtggtggtggacgtgagccacgaagaccctgaggtcaagttcaactggtacgtggacggcgtggaggtgcataatgccaagacaaagccgcgggaggagcagtacaacagcacgtaccgtgtggtcagcgtcctcaccgtcctgcaccaggactggctgaatggcaaggagtacaagtgcaaggtctccaacaaagccctcccagcccccatcgagaaaaccatctccaaagccaaagggcagccccgagaaccacaggtgtacaccctgcccccatcccgggaggagatgaccaagaaccaggtcagcctgacctgcctggtcaaaggcttctatcccagcgacatcgccgtggagtgggagagcaatgggcagccggagaacaactacaagaccacgcctcccgtgctggactccgacggctccttcttcctctacagcaagctcaccgtggacaagagcaggtggcagcaggggaacgtcttctcatgctccgtgatgcatgaggctctgcacaaccactacacgcagaagagcctctccctgtctccgggtaaa

SEQ ID NO: 56 - DNA, 639 bp, synthetic construct; identical to SEQ ID NO: 54
  source 1..639: mol_type = other DNA